European Patent Application EP 4 302 836 A1, published January 10, 2024. Title: Antibodies against snake toxins causing muscle and/or tissue damage. Applicant: Danmarks Tekniske Universitet. The sequence listing filed with the application follows.

SEQUENCE LISTING (28 sequences)

SEQ ID NO: 1 - protein, 121 aa, Bothrops asper
  SITE 1..121: note = Polypeptide sequence of Myotoxin II (Basic phospholipase A2homolog 2, uniprot ID P24605)
SLFELGKMILQETGKNPAKSYGAYGCNCGVLGRGKPKDATDRCCYVHKCCYKKLTGCNPKKDRYSYSWKDKTIVCGENNSCLKELCECDKAVAICLRENLNTYNKKYRYYLKPLCKKADAC

SEQ ID NO: 2 - protein, 8 aa, Homo sapiens
  SITE 1..8: note = Polypeptide sequence of variable heavy chain CDR1 (CDR-H1) ofantibodies TPL0039_05_B12, TPL0039_05_F04, TPL0039_05_G08,TPL0039_05_B04, TPL0039_05_A03.
GFTFSSYG

SEQ ID NO: 3 - protein, 8 aa, Homo sapiens
  SITE 1..8: note = Polypeptide sequence of variable heavy chain CDR2 (CDR-H2) ofantibodies TPL0039_05_B12, TPL0039_05_F04, TPL0039_05_G08,TPL0039_05_B04, TPL0039_05_A03
ISYDGSNK

SEQ ID NO: 4 - protein, 11 aa, Homo sapiens
  SITE 1..11: note = Polypeptide sequence of variable heavy chain CDR3 (CDR-H3) ofantibody TPL0039_05_B12
AGWTEGDAFDI

SEQ ID NO: 5 - protein, 8 aa, Homo sapiens
  SITE 1..8: note = Polypeptide sequence of variable light chain CDR1 (CDR-L1) ofantibodies TPL0039_05_B12, TPL0039_05_F04, TPL0039_05_G08,TPL0039_05_A03.
SGSIASNY

SEQ ID NO: 6 - skipped

SEQ ID NO: 7 - protein, 9 aa, Homo sapiens
  SITE 1..9: note = Polypeptide sequence of variable light chain CDR3 (CDR-L3) ofantibody TPL0039_05_B12, TPL0039_05_A03.
QSYDSSSVV

SEQ ID NO: 8 - protein, 10 aa, Homo sapiens
  SITE 1..10: note = Polypeptide sequence of variable heavy chain CDR3 (CDR-H3) ofantibody TPL0039_05_F04
AKDLEYSSSS

SEQ ID NO: 9 - skipped

SEQ ID NO: 10 - protein, 9 aa, Homo sapiens
  SITE 1..9: note = Polypeptide sequence of variable light chain CDR3 (CDR-L3) ofantibodies TPL0039_05_F04, TPL0039_05_G08, TPL0039_05_B04
QSYDSSTVV

SEQ ID NO: 11 - protein, 13 aa, Homo sapiens
  SITE 1..13: note = Polypeptide sequence of variable heavy chain CDR3 (CDR-H3) ofantibody TPL0039_05_G08
ARTNYDSGDAFDI

SEQ ID NO: 12 - protein, 11 aa, Homo sapiens
  SITE 1..11: note = Polypeptide sequence of variable heavy chain CDR3 (CDR-H3) ofantibody TPL0039_05_B04
ARVGENEAFDI

SEQ ID NO: 13 - protein, 8 aa, Homo sapiens
  SITE 1..8: note = Polypeptide sequence of variable light chain CDR1 (CDR-L1) ofantibody TPL0039_05_B04
SGSIARNY

SEQ ID NO: 14 - protein, 118 aa, Homo sapiens
  SITE 1..118: note = Polypeptide sequence of variable heavy chain of antibodyTPL0039_05_B12
EVQLVESGGGVVQPGRSLRLSCAASGFTFSSYGMHWVRQAPGKGLEWVAVISYDGSNKYYADSVKGRFTISRDNSKNTLYLQMNSLRAEDTAVYYCAGWTEGDAFDIWGQGTLVTVSS

SEQ ID NO: 15 - protein, 113 aa, Homo sapiens
  SITE 1..113: note = Polypeptide sequence of variable light chain of antibodyTPL0039_05_B12
NFMLTQPHSVSESPGKTVTISCTRSSGSIASNYVQWYQQRPGSAPSTVIYEDNRRPSGVPDRFSGSIDSASNSASLTISGLKTEDEADYYCQSYDSSSVVFGGGTKITVLGQP

SEQ ID NO: 16 - protein, 117 aa, Homo sapiens
  SITE 1..117: note = Polypeptide sequence of variable heavy chain of antibodyTPL0039_05_F04
QVQLVESGGGVVQPGRSPRLSCAASGFTFSSYGMHWVRQAPGKGLEWVAVISYDGSNKYYADSVKGRFTISRDNSKNTLYLQMNSLRAEDTAVYYCAKDLEYSSSSWGQGTLVTVSS

SEQ ID NO: 17 - protein, 113 aa, Homo sapiens
  SITE 1..113: note = Polypeptide sequence of variable light chain of antibodyTPL0039_05_F04
NFMLTQPHSVSESPGKTVTISCTRSSGSIASNYVQWFQQRPGSSPTTVIYEDDQRPSGVPDRFSGSIDSSSNSASLTISGLKTEDEATYFCQSYDSSTVVFGGGTKVTVLGQP

SEQ ID NO: 18 - protein, 120 aa, Homo sapiens
  SITE 1..120: note = Polypeptide sequence of variable heavy chain of antibodyTPL0039_05_G08
EVQLVESGGGVVQPGRSLRLSCAASGFTFSSYGMHWVRQAPGKGLEWVAVISYDGSNKYYADSVKGRFTISRDNSKNTLYLQMNSLRAEDTAVYYCARTNYDSGDAFDIWGQGTLVTVSS

SEQ ID NO: 19 - protein, 113 aa, Homo sapiens
  SITE 1..113: note = Polypeptide sequence of variable light chain of antibodyTPL0039_05_G08
NFMLTQPHSVSESPGKTVTISCTRSSGSIASNYVQWYQQRPGSSPTTVIYEDNQRPSGVPDRFSGSIDSSSNSASLTISGLKTEDEADYYCQSYDSSTVVFGGGTKLTVLGQP

SEQ ID NO: 20 - protein, 118 aa, Homo sapiens
  SITE 1..118: note = Polypeptide sequence of variable heavy chain of antibodyTPL0039_05_B04
EVQLLESGGGVVQPGRSLRLSCAASGFTFSSYGMHWVRQAPGKGLEWVAVISYDGSNKYYADSVKGRFTISRDNSKNTLYLQMNSLRAEDTAVYYCARVGENEAFDIWGQGTMVTVSS

SEQ ID NO: 21 - protein, 113 aa, Homo sapiens
  SITE 1..113: note = Polypeptide sequence of variable light chain of antibodyTPL0039_05_B04
NFMLTQPHSVSESPGKTVTISCTRSSGSIARNYVQWYQQRPGSAPTTVIYEDNQRPSGVPDRFSGSIDSSSNSASLTISGLKTEDEADYYCQSYDSSTVVFGGGTKLTVLGQP

SEQ ID NO: 22 - protein, 13 aa, Bothrops asper
  SITE 1..13: note = Polypeptide sequence of the B. asper Myotoxin II epitope
KKYRYYLKPLCKK

SEQ ID NO: 23 - protein, 12 aa, Homo sapiens
  SITE 1..12: note = Polypeptide sequence of variable heavy chain CDR3 (CDR-H3) ofantibody
ASTLQQLDAFDI

SEQ ID NO: 24 - protein, 119 aa, Homo sapiens
  SITE 1..119: note = Polypeptide sequence of variable heavy chain of antibodyTPL0039_05_A03.
QVQLVESGGGLAKPGRSLRLSCAVSGFTFSSYGMHWVRQAPGKGLEWVAVISYDGSNKYYADSVKGRFTISRDNSKNTLYLQMNSLRAEDTAVYYCASTLQQLDAFDIWGQGTMVTVSS

SEQ ID NO: 25 - protein, 113 aa, Homo sapiens
  SITE 1..113: note = Polypeptide sequence of variable light chain of antibodyTPL0039_05_A03
NFMLTQPHSVSESPGKTITISCTRSSGSIASNYVQWYQQRPGSVPTPVIYEDDRRPSGVPDRFSGSIDSSSNSASLTISGLKTEDEADYYCQSYDSSSVVFGGGTKITVLGQP

SEQ ID NO: 26 - DNA, 24 bp, synthetic construct
  misc_feature 1..24: note = Primer for sequencing
  misc_feature 1..24: note = Polynucleotide sequence of the S10b primer
  source 1..24: mol_type = other DNA
ggctttgttagcagccggatctca

SEQ ID NO: 27 - DNA, 25 bp, synthetic construct
  misc_feature 1..25: note = Primer for sequencing
  misc_feature 1..25: note = Polynucleotide sequence of the pINT VH Seq Fwd primer
  source 1..25: mol_type = other DNA
tggagctgtatcatcctcttcttgg

SEQ ID NO: 28 - DNA, 33 bp, synthetic construct
  misc_feature 1..33: note = Primer for sequencing
  misc_feature 1..33: note = Polynucleotide sequence of the pINT VL lambda seq R primer
  source 1..33: mol_type = other DNA
actccggctttcactggggagctgtctgccttc